European Patent Application EP 4 775 228 A1, published July 15, 2026. Title: METHODS FOR IMPROVING CARDIAC FUNCTION IN ARRHYTHMOGENIC RIGHT VENTRICULAR CARDIOMYOPATHY TYPE 5. Applicant: Centro Nacional de Investigaciones Cardiovasculares Carlos III (F.S.P.). The sequence listing filed with the application follows.

SEQUENCE LISTING (22 sequences)

SEQ ID NO: 1 - DNA, 1203 bp, Homo sapiens
  source 1..1203: mol_type = genomic DNA; note = Wild type nucleotidic sequence of TMEM43; note (original language) = Secuencia nucleotidica de TMEM43 salvaje
atggccgcgaattattccagtaccagtacccggagagaacatgtcaaagttaaaaccagctcccagccaggcttcctggaacggctgagcgagacctcgggtgggatgtttgtggggctcatggccttcctgctctccttctacctaattttcaccaatgagggccgcgcattgaagacggcaacctcattggctgaggggctctcgcttgtggtgtctcccgacagcatccacagtgtggctccggagaatgaaggaaggctggtgcacatcattggcgccttacggacatccaagcttttgtctgatccaaactatggggtccatcttccggctgtgaaactgcggaggcacgtggagatgtaccaatgggtagaaactgaggagtccagggagtacaccgaggatgggcaggtgaagaaggagacgaggtattcctacaacactgaatggaggtcagaaatcatcaacagcaaaaacttcgaccgagagattggccacaaaaaccccagtgccatggcagtggagtcattcatggcaacagccccctttgtccaaattggcaggtttttcctctcgtcaggcctcatcgacaaagtcgacaacttcaagtccctgagcctatccaagctggaggaccctcatgtggacatcattcgccgtggagactttttctaccacagcgaaaatcccaagtatccagaggtgggagacttgcgtgtctccttttcctatgctggactgagcggcgatgaccctgacctgggcccagctcacgtggtcactgtgattgcccggcagcggggtgaccagctagtcccattctccaccaagtctggggataccttactgctcctgcaccacggggacttctcagcagaggaggtgtttcatagagaactaaggagcaactccatgaagacctggggcctgcgggcagctggctggatggccatgttcatgggcctcaaccttatgacacggatcctctacaccttggtggactggtttcctgttttccgagacctggtcaacattggcctgaaagcctttgccttctgtgtggccacctcgctgaccctgctgaccgtggcggctggctggctcttctaccgacccctgtgggccctcctcattgccggcctggcccttgtgcccatccttgttgctcggacacgggtgccagccaaaaagttggagtga

SEQ ID NO: 2 - protein, 400 aa, Homo sapiens
  source 1..400: note = Protein sequence wild type TMEM43; note (original language) = Secuencia proteica TMEM43 salvaje
MAANYSSTSTRREHVKVKTSSQPGFLERLSETSGGMFVGLMAFLLSFYLIFTNEGRALKTATSLAEGLSLVVSPDSIHSVAPENEGRLVHIIGALRTSKLLSDPNYGVHLPAVKLRRHVEMYQWVETEESREYTEDGQVKKETRYSYNTEWRSEIINSKNFDREIGHKNPSAMAVESFMATAPFVQIGRFFLSSGLIDKVDNFKSLSLSKLEDPHVDIIRRGDFFYHSENPKYPEVGDLRVSFSYAGLSGDDPDLGPAHVVTVIARQRGDQLVPFSTKSGDTLLLLHHGDFSAEEVFHRELRSNSMKTWGLRAAGWMAMFMGLNLMTRILYTLVDWFPVFRDLVNIGLKAFAFCVATSLTLLTVAAGWLFYRPLWALLIAGLALVPILVARTRVPAKKLE

SEQ ID NO: 3 - DNA, 1203 bp, synthetic construct
  source 1..1203: mol_type = other DNA; note = Mutant TMEM43 S358L; note (original language) = Mutante TMEM43 S358L; organism (original language) = Constructo sintético
atggccgcgaattattccagtaccagtacccggagagaacatgtcaaagttaaaaccagctcccagccaggcttcctggaacggctgagcgagacctcgggtgggatgtttgtggggctcatggccttcctgctctccttctacctaattttcaccaatgagggccgcgcattgaagacggcaacctcattggctgaggggctctcgcttgtggtgtctcccgacagcatccacagtgtggctccggagaatgaaggaaggctggtgcacatcattggcgccttacggacatccaagcttttgtctgatccaaactatggggtccatcttccggctgtgaaactgcggaggcacgtggagatgtaccaatgggtagaaactgaggagtccagggagtacaccgaggatgggcaggtgaagaaggagacgaggtattcctacaacactgaatggaggtcagaaatcatcaacagcaaaaacttcgaccgagagattggccacaaaaaccccagtgccatggcagtggagtcattcatggcaacagccccctttgtccaaattggcaggtttttcctctcgtcaggcctcatcgacaaagtcgacaacttcaagtccctgagcctatccaagctggaggaccctcatgtggacatcattcgccgtggagactttttctaccacagcgaaaatcccaagtatccagaggtgggagacttgcgtgtctccttttcctatgctggactgagcggcgatgaccctgacctgggcccagctcacgtggtcactgtgattgcccggcagcggggtgaccagctagtcccattctccaccaagtctggggataccttactgctcctgcaccacggggacttctcagcagaggaggtgtttcatagagaactaaggagcaactccatgaagacctggggcctgcgggcagctggctggatggccatgttcatgggcctcaaccttatgacacggatcctctacaccttggtggactggtttcctgttttccgagacctggtcaacattggcctgaaagcctttgccttctgtgtggccaccttgctgaccctgctgaccgtggcggctggctggctcttctaccgacccctgtgggccctcctcattgccggcctggcccttgtgcccatccttgttgctcggacacgggtgccagccaaaaagttggagtga

SEQ ID NO: 4 - protein, 399 aa, synthetic construct
  source 1..399: note = Mutant TMEM43 S358L; note (original language) = Mutante TMEM43 S358L; organism (original language) = Constructo sintetico
MAANYSSTSTRREHVKVKTSSQPGFLERLSETSGGMFVGLMAFLLSFYLIFTNEGRALKTATSLAEGLSLVVSPDSIHSVAPENEGRLVHIIGALRTSKLLSDPNYGVHLPAVKLRRHVEMYQWVETEESREYTEDGQVKKETRYSYNTEWRSEIINSKNFDREIGHKNPSAMAVESFMATAPFVQIGRFFLSSGLIDKVDNFKSLSLSKLEDPHVDIIRRGDFFYHSENPKYPEVGDLRVSFSYAGLSGDDPDLGPAHVVTVIARQRGDQLVPFSTKSGDTLLLLHHGDFSAEEVFHRELRSNSMKTWGLRAAGWMAMFMGLNLMTRILYTLVDWFPVFRDLVNIGLKAFAFCVATLLTLLTVAAGWLFYRPLWALLIAGLALVPILVARTRVPAKKL

SEQ ID NO: 5 - DNA, 1203 bp, synthetic construct
  source 1..1203: mol_type = other DNA; note = TMEM43 codon-optimized; note (original language) = Codones optimizados TMEM43; organism (original language) = Constructo sintetico
atggccgccaactactcctctacctccaccaggagagagcacgtcaaggtgaagacatcctcccagcccggcttcctggagaggctgagtgaaacctctggcggcatgtttgtgggcctgatggccttcctgctgtctttttacctgatctttacaaacgagggcagggccctgaagacagccacctctctggctgaaggccttagcctggtcgtgtccccagattctatccacagcgtggctcctgagaacgagggaagattggtgcacattatcggggccctgcgcacctccaaactgctgagtgaccccaactacggcgtgcacctccccgccgtgaaactgagacgccatgtggagatgtaccagtgggtcgagaccgaggaaagccgagagtataccgaggatggccaggtgaagaaggagactcgctacagctacaacaccgagtggagatccgagatcatcaactccaagaacttcgacagggagatcggacataagaacccatcagccatggccgtggagtctttcatggccactgctcctttcgtgcagatcggccggttcttcctgagctctggcctgatcgacaaggtggacaacttcaagagcctgtccctgtctaagctggaggatcctcacgtggatatcatccgcaggggagatttcttctaccacagcgagaacccaaaatatcctgaggtgggagacctgagagtgagcttctcctacgccggcctgagcggcgatgaccccgatctgggccccgcccacgtggtgacagtgatcgcccgacagcgcggcgatcagctggtgccattcagcaccaagagcggtgacaccctgctgctgctgcaccatggggatttttccgctgaggaggtgttccacagggagctgcggagcaatagtatgaagacatgggggctgagggccgcaggctggatggccatgttcatgggactgaacctgatgacaaggatcctgtacacactggtggactggtttcctgtgttcagagacctggtgaatattggcctgaaggccttcgctttctgcgtggccaccagcctgaccctgctgaccgtggccgccgggtggctgttctacaggccactctgggctctgctgatcgccgggctggccctggtccctatcctcgtggctagaactagagtgccagctaagaagctggaatga

SEQ ID NO: 6 - DNA, 1203 bp, synthetic construct
  source 1..1203: mol_type = other DNA; note = codon optimized TMEM43-UF; note (original language) = Codones optimizados TMEM43-UF; organism (original language) = Constructo sintetico
atggccgcaaactactcaagcacctctacacgacgggagcacgtcaaagtgaaaacctcatctcagcctggattcctggagcgactgagcgagacatccggcggcatgttcgtgggcctgatggccttcctgctgagcttttacctgatcttcaccaacgagggcagggccctgaagacagccacatctctggccgagggcctgagcctggtggtgtctcccgacagcatccactctgtggcacctgagaatgagggcaggctggtgcacatcatcggcgccctgcgcacatccaagctgctgtctgatcctaattatggagtgcacctgccagcagtgaagctgcggagacacgtggagatgtaccagtgggtggagacagaggagagccgcgagtataccgaggacggccaggtgaagaaggagacacggtactcctataacaccgagtggagaagcgagatcatcaactccaagaattttgatagggagatcggccacaagaatccatccgccatggccgtggagtcttttatggcaacagcacccttcgtgcagattggccgcttctttctgagctccggcctgatcgacaaggtggataacttcaagtctctgagcctgtccaagctggaggacccccacgtggatatcatcaggcgcggcgacttcttttaccactctgagaatcccaagtatcctgaagtgggcgatctgcgggtgtcttttagctatgcaggcctgtctggcgacgatccagacctgggacctgcacacgtggtgacagtgatcgcaagacagagaggcgatcagctggtgcctttctctacaaagtctggcgacaccctgctgctgctgcaccacggcgacttcagcgccgaggaggtgttccacagggagctgcgctccaactctatgaagacatggggcctgagagcagcaggatggatggccatgtttatgggcctgaatctgatgacacggatcctgtacaccctggtggactggttccccgtgttccgggacctggtgaatatcggcctgaaggccttcgccttttgcgtggccacctccctgacactgctgacagtggcagcaggatggctgttctatagaccactgtgggccctgctgatcgccggcctggctctggtcccaatcctggtggcaagaactcgggtccctgctaagaaactggaataa

SEQ ID NO: 7 - DNA, 26 bp, synthetic construct
  source 1..26: mol_type = other DNA; note = human TMEM43 forward primer; note (original language) = cebador sentido TMEM43 humano; organism (original language) = Constructo sintetico
tcccaagtatccagaggtgggagact

SEQ ID NO: 8 - DNA, 19 bp, synthetic construct
  source 1..19: mol_type = other DNA; note = human TMEM43 reverse primer; note (original language) = cebador antisentido TMEM43 humano; organism (original language) = Constructo sintetico
aggccggcaatgaggaggg

SEQ ID NO: 9 - DNA, 18 bp, synthetic construct
  source 1..18: mol_type = other DNA; note = LOX forward primer; note (original language) = Cebador LOX sentido; organism (original language) = Constructo sintetico
gctgcggaagaaaactgc

SEQ ID NO: 10 - DNA, 21 bp, synthetic construct
  misc_feature 1..21
  source 1..21: mol_type = other DNA; note = LOX forward primer; note (original language) = Cebador LOX antisentido; organism (original language) = Constructo sintetico
ccttggttcttcactctttgc

SEQ ID NO: 11 - DNA, 18 bp, synthetic construct
  source 1..18: mol_type = other DNA; note = POSTN forward primer; note (original language) = cebador POSTN sentido; organism (original language) = Constructo sintetico
aacgtctgtgccctccag

SEQ ID NO: 12 - DNA, 20 bp, synthetic construct
  source 1..20: mol_type = other DNA; note = Primer POSTN reverse; note (original language) = Cebador POSTN antisentido; organism (original language) = Constructo sintetico
agcctttcatcccttccatt

SEQ ID NO: 13 - DNA, 20 bp, synthetic construct
  source 1..20: mol_type = other DNA; note = Primer COL1A1 forward; note (original language) = Cebador COL1A1 sentido; organism (original language) = Constructo sintético
gtgccactctgactggaaga

SEQ ID NO: 14 - DNA, 20 bp, synthetic construct
  source 1..20: mol_type = other DNA; note = Primer COL1A1 reverse; note (original language) = Cebador COL1A1 antisentido; organism (original language) = Constructo sintetico
ctgacctgtctccatgttgc

SEQ ID NO: 15 - DNA, 20 bp, synthetic construct
  source 1..20: mol_type = other DNA; note = Primer COL3A1 forward; note (original language) = Cebador sentido COL3A1; organism (original language) = Constructo sintetico
cacccttcttcatcccactc

SEQ ID NO: 16 - DNA, 20 bp, synthetic construct
  source 1..20: mol_type = other DNA; note = Primer COL3A1 reverse; note (original language) = Cebador antisentido COL3A1; organism (original language) = Constructo sintetico
atgtcatcgcaaaggacaga

SEQ ID NO: 17 - DNA, 20 bp, synthetic construct
  source 1..20: mol_type = other DNA; note = Primer ACTA1 forward; note (original language) = Cebador sentido ACTA1; organism (original language) = Constructo sintetico
gaccacagctgaacgtgaga

SEQ ID NO: 18 - DNA, 22 bp, synthetic construct
  source 1..22: mol_type = other DNA; note = Primer ACTA1 reverse; note (original language) = Cebador antisentido ACTA1; organism (original language) = Constructo sintetico
tgttgtaggtggtctcatggat

SEQ ID NO: 19 - DNA, 21 bp, synthetic construct
  source 1..21: mol_type = other DNA; note = Primer luciferase forward; note (original language) = Cebador sentido luciferasa; organism (original language) = Constructo sintetico
tatcatggcctcgtgaaatcc

SEQ ID NO: 20 - DNA, 22 bp, synthetic construct
  source 1..22: mol_type = other DNA; note = Primer luciferase reverse; note (original language) = Cebador antisentido luciferasa; organism (original language) = Constructo sintetico
tcctgggtccgattcaataaac

SEQ ID NO: 21 - DNA, 413 bp, Gallus gallus
  source 1..413: mol_type = genomic DNA; note = cardiac troponin T promoter (cTnT); note (original language) = Promotor de la troponina T cardiaca (cTnT)
gggataaaagcagtctgggctttcacatgacagcatctggggctgcggcagagggtcgggtccgaagcgctgccttatcagcgtccccagccctgggaggtgacagctggctggcttgtgtcagcccctcgggcactcacgtatctccgtccgacgggtttaaaatagcaaaactctgaggccacacaatagcttgggcttatatgggctcctgtgggggaagggggagcacggagggggccggggccgctgctgccaaaatagcagctcacaagtgttgcattcctctctgggcgccgggcacattcctgctggctctgcccgccccggggtgggcgccggggggaccttaaagcctctgccccccaaggagcccttcccagacagccgccggcacccaccgctccgtggga

SEQ ID NO: 22 - DNA, 222 bp, synthetic construct
  source 1..222: mol_type = other DNA; note = SV40 late polyA signal; note (original language) = Señal poliA de SV40; organism (original language) = Constructo sintetico
cagacatgataagatacattgatgagtttggacaaaccacaactagaatgcagtgaaaaaaatgctttatttgtgaaatttgtgatgctattgctttatttgtaaccattataagctgcaataaacaagttaacaacaacaattgcattcattttatgtttcaggttcagggggaggtgtgggaggttttttaaagcaagtaaaacctctacaaatgtggta